European Patent Specification EP 3 298 140 B1, published April 24, 2024. Title: Compositions for Treating Pathological Calcification Conditions, and Methods Using Same. Applicant: Yale University Braddock, Demetrios Albright, Ronald. The sequence listing filed with the application follows.

SEQUENCE LISTING (30 sequences)

SEQ ID NO: 1 - protein, 925 aa, Homo sapiens
MERDGCAGGGSRGGEGGRAPREGPAGNGRDRGRSHAAEAPGDPQAAASLLAPMDVGEEPLEKAARARTAKDPNTYKVLSLVLSVCVLTTILGCIFGLKPSCAKEVKSCKGRCFERTFGNCRCDAACVELGNCCLDYQETCIEPEHIWTCNKFRCGEKRLTRSLCACSDDCKDKGDCCINYSSVCQGEKSWVEEPCESINEPQCPAGFETPPTLLFSLDGFRAEYLHTWGGLLPVISKLKKCGTYTKNMRPVYPTKTFPNHYSIVTGLYPESHGIIDNKMYDPKMNASFSLKSKEKFNPEWYKGEPIWVTAKYQGLKSGTFFWPGSDVEINGIFPDIYKMYNGSVPFEERILAVLQWLQLPKDERPHFYTLYLEEPDSSGHSYGPVSSEVIKALQRVDGMVGMLMDGLKELNLHRCLNLILISDHGMEQGSCKKYIYLNKYLGDVKNIKVIYGPAARLRPSDVPDKYYSFNYEGIARNLSCREPNQHFKPYLKHFLPKRLHFAKSDRIEPLTFYLDPQWQLALNPSERKYCGSGFHGSDNVFSNMQALFVGYGPGFKHGIEADTFENIEVYNLMCDLLNLTPAPNNGTHGSLNHLLKNPVYTPKHPKEVHPLVQCPFTRNPRDNLGCSCNPSILPIEDFQTQFNLTVAEEKIIKHETLPYGRPRVLQKENTICLLSQHQFMSGYSQDILMPLWTSYTVDRNDSFSTEDFSNCLYQDFRIPLSPVHKCSFYKNNTKVSYGFLSPPQLNKNSSGIYSEALLTTNIVPMYQSFQVIWRYFHDTLLRKYAEERNGVNVVSGPVFDFDYDGRCDSLENLRQKRRVIRNQEILIPTHFFIVLTSCKDTSQTPLHCENLDTLAFILPHRTDNSESCVHGKHDSSWVEELLMLHRARITDVEHITGLSFYQQRKEPVSDILKLKTHLPTFSQED

SEQ ID NO: 2 - protein, 888 aa, Homo sapiens
MARRSSFQSCQIISLFTFAVGVNICLGFTAHRIKRAEGWEEGPPTVLSDSPWTNISGSCKGRCFELQEAGPPDCRCDNLCKSYTSCCHDFDELCLKTARGWECTKDRCGEVRNEENACHCSEDCLARGDCCTNYQVVCKGESHWVDDDCEEIKAAECPAGFVRPPLIIFSVDGFRASYMKKGSKVMPNIEKLRSCGTHSPYMRPVYPTKTFPNLYTLATGLYPESHGIVGNSMYDPVFDATFHLRGREKFNHRWWGGQPLWITATKQGVKAGTFFWSVVIPHERRILTILQWLTLPDHERPSVYAFYSEQPDFSGHKYGPFGPEMTNPLREIDKIVGQLMDGLKQLKLHRCVNVIFVGDHGMEDVTCDRTEFLSNYLTNVDDITLVPGTLGRIRSKFSNNAKYDPKAIIANLTCKKPDQHFKPYLKQHLPKRLHYANNRRIEDIHLLVERRWHVARKPLDVYKKPSGKCFFQGDHGFDNKVNSMQTVFVGYGSTFKYKTKVPPFENIELYNVMCDLLGLKPAPNNGTHGSLNHLLRTNTFRPTMPEEVTRPNYPGIMYLQSDFDLGCTCDDKVEPKNKLDELNKRLHTKGSTEAETRKFRGSRNENKENINGNFEPRKERHLLYGRPAVLYRTRYDILYHTDFESGYSEIFLMPLWTSYTVSKQAEVSSVPDHLTSCVRPDVRVSPSFSQNCLAYKNDKQMSYGFLFPPYLSSSPEAKYDAFLVTNMVPMYPAFKRVWNYFQRVLVKKYASERNGVNVISGPIFDYDYDGLHDTEDKIKQYVEGSSIPVPTHYYSIITSCLDFTQPADKCDGPLSVSSFILPHRPDNEESCNSSEDESKWVEELMKMHTARVRDIEHLTSLDFFRKTSRSYPEILTLKTYLHTYESEI

SEQ ID NO: 3 - protein, 453 aa, Homo sapiens
MKLLVILLFSGLITGFRSDSSSSLPPKLLLVSFDGFRADYLKNYEFPHLQNFIKEGVLVEHVKNVFITKTFPNHYSIVTGLYEESHGIVANSMYDAVTKKHFSDSNDKDPFWWNEAVPIWVTNQLQENRSSAAAMWPGTDVPIHDTISSYFMNYNSSVSFEERLNNITMWLNNSNPPVTFATLYWEEPDASGHKYGPEDKENMSRVLKKIDDLIGDLVQRLKMLGLWENLNVIITSDHGMTQCSQDRLINLDSCIDHSYYTLIDLSPVAAILPKINRTEVYNKLKNCSPHMNVYLKEDIPNRFYYQHNDRIQPIILVADEGWTIVLNESSQKLGDHGYDNSLPSMHPFLAAHGPAFHKGYKHSTINIVDIYPMMCHILGLKPHPNNGTFGHTKCLLVDQWCINLPEAIAIVIGSLLVLTMLTCLIIIMQNRLSVPRPFSRLQLQEDDDDPLIG

SEQ ID NO: 4 - protein, 3 aa, Artificial Sequence
  chemically synthesized
  REPEAT (1)..(3): the tripeptide is present n times, wherein n is integer ranging from 1 to 10
DSS

SEQ ID NO: 5 - protein, 3 aa, Artificial Sequence
  chemically synthesized
  REPEAT (1)..(3): the tripeptide is present n times, wherein n is an integer ranging from 1 to 10
ESS

SEQ ID NO: 6 - protein, 3 aa, Artificial Sequence
  chemically synthesized
  REPEAT (1)..(3): the tripeptide is present n times, wherein n is integer ranging from 1 to 10
RQQ

SEQ ID NO: 7 - protein, 2 aa, Artificial Sequence
  chemically synthesized
  REPEAT (1)..(2): the dipeptide is present n times, wherein n is integer ranging from 1 to 10
KR

SEQ ID NO: 8 - protein, 1 aa, Artificial Sequence
  chemically synthesized
  REPEAT (1)..(1): the amino acid is present n times, wherein n is integer ranging from 1 to 10
R

SEQ ID NO: 9 - protein, 16 aa, Artificial Sequence
  chemically synthesized
DSSSEEKFLRRIGRFG

SEQ ID NO: 10 - protein, 12 aa, Artificial Sequence
  chemically synthesized
EEEEEEEPRGDT

SEQ ID NO: 11 - protein, 12 aa, Artificial Sequence
  chemically synthesized
APWHLSSQYSRT

SEQ ID NO: 12 - protein, 12 aa, Artificial Sequence
  chemically synthesized
STLPIPHEFSRE

SEQ ID NO: 13 - protein, 12 aa, Artificial Sequence
  chemically synthesized
VTKHLNQISQSY

SEQ ID NO: 14 - protein, 1 aa, Artificial Sequence
  chemically sysnthesized
  REPEAT (1)..(1): the amino acid is present m times, wherein m is an integer ranging from 1 to 15
E

SEQ ID NO: 15 - protein, 925 aa, Artificial Sequence
  chemically synthesized
MERDGCAGGGSRGGEGGRAPREGPAGNGRDRGRSHAAEAPGDPQAAASLLAPMDVGEEPLEKAARARTAKDPNTYKIISLFTFAVGVNICLGFTAGLKPSCAKEVKSCKGRCFERTFGNCRCDAACVELGNCCLDYQETCIEPEHIWTCNKFRCGEKRLTRSLCACSDDCKDKGDCCINYSSVCQGEKSWVEEPCESINEPQCPAGFETPPTLLFSLDGFRAEYLHTWGGLLPVISKLKKCGTYTKNMRPVYPTKTFPNHYSIVTGLYPESHGIIDNKMYDPKMNASFSLKSKEKFNPEWYKGEPIWVTAKYQGLKSGTFFWPGSDVEINGIFPDIYKMYNGSVPFEERILAVLQWLQLPKDERPHFYTLYLEEPDSSGHSYGPVSSEVIKALQRVDGMVGMLMDGLKELNLHRCLNLILISDHGMEQGSCKKYIYLNKYLGDVKNIKVIYGPAARLRPSDVPDKYYSFNYEGIARNLSCREPNQHFKPYLKHFLPKRLHFAKSDRIEPLTFYLDPQWQLALNPSERKYCGSGFHGSDNVFSNMQALFVGYGPGFKHGIEADTFENIEVYNLMCDLLNLTPAPNNGTHGSLNHLLKNPVYTPKHPKEVHPLVQCPFTRNPRDNLGCSCNPSILPIEDFQTQFNLTVAEEKIIKHETLPYGRPRVLQKENTICLLSQHQFMSGYSQDILMPLWTSYTVDRNDSFSTEDFSNCLYQDFRIPLSPVHKCSFYKNNTKVSYGFLSPPQLNKNSSGIYSEALLTTNIVPMYQSFQVIWRYFHDTLLRKYAEERNGVNVVSGPVFDFDYDGRCDSLENLRQKRRVIRNQEILIPTHFFIVLTSCKDTSQTPLHCENLDTLAFILPHRTDNSESCVHGKHDSSWVEELLMLHRARITDVEHITGLSFYQQRKEPVSDILKLKTHLPTFSQED

SEQ ID NO: 16 - protein, 1155 aa, Artificial Sequence
  chemically synthesized
MERDGCAGGGSRGGEGGRAPREGPAGNGRDRGRSHAAEAPGDPQAAASLLAPMDVGEEPLEKAARARTAKDPNTYKIISLFTFAVGVNICLGFTAGLKPSCAKEVKSCKGRCFERTFGNCRCDAACVELGNCCLDYQETCIEPEHIWTCNKFRCGEKRLTRSLCACSDDCKDKGDCCINYSSVCQGEKSWVEEPCESINEPQCPAGFETPPTLLFSLDGFRAEYLHTWGGLLPVISKLKKCGTYTKNMRPVYPTKTFPNHYSIVTGLYPESHGIIDNKMYDPKMNASFSLKSKEKFNPEWYKGEPIWVTAKYQGLKSGTFFWPGSDVEINGIFPDIYKMYNGSVPFEERILAVLQWLQLPKDERPHFYTLYLEEPDSSGHSYGPVSSEVIKALQRVDGMVGMLMDGLKELNLHRCLNLILISDHGMEQGSCKKYIYLNKYLGDVKNIKVIYGPAARLRPSDVPDKYYSFNYEGIARNLSCREPNQHFKPYLKHFLPKRLHFAKSDRIEPLTFYLDPQWQLALNPSERKYCGSGFHGSDNVFSNMQALFVGYGPGFKHGIEADTFENIEVYNLMCDLLNLTPAPNNGTHGSLNHLLKNPVYTPKHPKEVHPLVQCPFTRNPRDNLGCSCNPSILPIEDFQTQFNLTVAEEKIIKHETLPYGRPRVLQKENTICLLSQHQFMSGYSQDILMPLWTSYTVDRNDSFSTEDFSNCLYQDFRIPLSPVHKCSFYKNNTKVSYGFLSPPQLNKNSSGIYSEALLTTNIVPMYQSFQVIWRYFHDTLLRKYAEERNGVNVVSGPVFDFDYDGRCDSLENLRQKRRVIRNQEILIPTHFFIVLTSCKDTSQTPLHCENLDTLAFILPHRTDNSESCVHGKHDSSWVEELLMLHRARITDVEHITGLSFYQQRKEPVSDILKLKTHLPTFSQEDLINDKTHTCPPCPAPELLGGPSVFLFPPKPKDTLMISRTPEVTCVVVDVSHEDPEVKFNWYVDGVEVHNAKTKPREEQYNSTYRVVSVLTVLHQDWLNGKEYKCKVSNKALPAPIEKTISKAKGQPREPQVYTLPPSREEMTKNQVSLTCLVKGFYPSDIAVEWESNGQPENNYKTTPPVLDSDGSFFLYSKLTVDKSRWQQGNVFSCSVMHEALHNHYTQKSLSLSPGK

SEQ ID NO: 17 - protein, 852 aa, Artificial Sequence
  chemically synthesized
MRGPAVLLTVALATLLAPGAGAGLKPSCAKEVKSCKGRCFERTFGNCRCDAACVELGNCCLDYQETCIEPEHIWTCNKFRCGEKRLTRSLCACSDDCKDKGDCCINYSSVCQGEKSWVEEPCESINEPQCPAGFETPPTLLFSLDGFRAEYLHTWGGLLPVISKLKKCGTYTKNMRPVYPTKTFPNHYSIVTGLYPESHGIIDNKMYDPKMNASFSLKSKEKFNPEWYKGEPIWVTAKYQGLKSGTFFWPGSDVEINGIFPDIYKMYNGSVPFEERILAVLQWLQLPKDERPHFYTLYLEEPDSSGHSYGPVSSEVIKALQRVDGMVGMLMDGLKELNLHRCLNLILISDHGMEQGSCKKYIYLNKYLGDVKNIKVIYGPAARLRPSDVPDKYYSFNYEGIARNLSCREPNQHFKPYLKHFLPKRLHFAKSDRIEPLTFYLDPQWQLALNPSERKYCGSGFHGSDNVFSNMQALFVGYGPGFKHGIEADTFENIEVYNLMCDLLNLTPAPNNGTHGSLNHLLKNPVYTPKHPKEVHPLVQCPFTRNPRDNLGCSCNPSILPIEDFQTQFNLTVAEEKIIKHETLPYGRPRVLQKENTICLLSQHQFMSGYSQDILMPLWTSYTVDRNDSFSTEDFSNCLYQDFRIPLSPVHKCSFYKNNTKVSYGFLSPPQLNKNSSGIYSEALLTTNIVPMYQSFQVIWRYFHDTLLRKYAEERNGVNVVSGPVFDFDYDGRCDSLENLRQKRRVIRNQEILIPTHFFIVLTSCKDTSQTPLHCENLDTLAFILPHRTDNSESCVHGKHDSSWVEELLMLHRARITDVEHITGLSFYQQRKEPVSDILKLKTHLPTFSQED

SEQ ID NO: 18 - protein, 1082 aa, Artificial Sequence
  chemically synthesized
MRGPAVLLTVALATLLAPGAGAGLKPSCAKEVKSCKGRCFERTFGNCRCDAACVELGNCCLDYQETCIEPEHIWTCNKFRCGEKRLTRSLCACSDDCKDKGDCCINYSSVCQGEKSWVEEPCESINEPQCPAGFETPPTLLFSLDGFRAEYLHTWGGLLPVISKLKKCGTYTKNMRPVYPTKTFPNHYSIVTGLYPESHGIIDNKMYDPKMNASFSLKSKEKFNPEWYKGEPIWVTAKYQGLKSGTFFWPGSDVEINGIFPDIYKMYNGSVPFEERILAVLQWLQLPKDERPHFYTLYLEEPDSSGHSYGPVSSEVIKALQRVDGMVGMLMDGLKELNLHRCLNLILISDHGMEQGSCKKYIYLNKYLGDVKNIKVIYGPAARLRPSDVPDKYYSFNYEGIARNLSCREPNQHFKPYLKHFLPKRLHFAKSDRIEPLTFYLDPQWQLALNPSERKYCGSGFHGSDNVFSNMQALFVGYGPGFKHGIEADTFENIEVYNLMCDLLNLTPAPNNGTHGSLNHLLKNPVYTPKHPKEVHPLVQCPFTRNPRDNLGCSCNPSILPIEDFQTQFNLTVAEEKIIKHETLPYGRPRVLQKENTICLLSQHQFMSGYSQDILMPLWTSYTVDRNDSFSTEDFSNCLYQDFRIPLSPVHKCSFYKNNTKVSYGFLSPPQLNKNSSGIYSEALLTTNIVPMYQSFQVIWRYFHDTLLRKYAEERNGVNVVSGPVFDFDYDGRCDSLENLRQKRRVIRNQEILIPTHFFIVLTSCKDTSQTPLHCENLDTLAFILPHRTDNSESCVHGKHDSSWVEELLMLHRARITDVEHITGLSFYQQRKEPVSDILKLKTHLPTFSQEDLINDKTHTCPPCPAPELLGGPSVFLFPPKPKDTLMISRTPEVTCVVVDVSHEDPEVKFNWYVDGVEVHNAKTKPREEQYNSTYRVVSVLTVLHQDWLNGKEYKCKVSNKALPAPIEKTISKAKGQPREPQVYTLPPSREEMTKNQVSLTCLVKGFYPSDIAVEWESNGQPENNYKTTPPVLDSDGSFFLYSKLTVDKSRWQQGNVFSCSVMHEALHNHYTQKSLSLSPGK

SEQ ID NO: 19 - protein, 849 aa, Artificial Sequence
  chemically synthesized
MRGPAVLLTVALATLLAPGAGAPSCAKEVKSCKGRCFERTFGNCRCDAACVELGNCCLDYQETCIEPEHIWTCNKFRCGEKRLTRSLCACSDDCKDKGDCCINYSSVCQGEKSWVEEPCESINEPQCPAGFETPPTLLFSLDGFRAEYLHTWGGLLPVISKLKKCGTYTKNMRPVYPTKTFPNHYSIVTGLYPESHGIIDNKMYDPKMNASFSLKSKEKFNPEWYKGEPIWVTAKYQGLKSGTFFWPGSDVEINGIFPDIYKMYNGSVPFEERILAVLQWLQLPKDERPHFYTLYLEEPDSSGHSYGPVSSEVIKALQRVDGMVGMLMDGLKELNLHRCLNLILISDHGMEQGSCKKYIYLNKYLGDVKNIKVIYGPAARLRPSDVPDKYYSFNYEGIARNLSCREPNQHFKPYLKHFLPKRLHFAKSDRIEPLTFYLDPQWQLALNPSERKYCGSGFHGSDNVFSNMQALFVGYGPGFKHGIEADTFENIEVYNLMCDLLNLTPAPNNGTHGSLNHLLKNPVYTPKHPKEVHPLVQCPFTRNPRDNLGCSCNPSILPIEDFQTQFNLTVAEEKIIKHETLPYGRPRVLQKENTICLLSQHQFMSGYSQDILMPLWTSYTVDRNDSFSTEDFSNCLYQDFRIPLSPVHKCSFYKNNTKVSYGFLSPPQLNKNSSGIYSEALLTTNIVPMYQSFQVIWRYFHDTLLRKYAEERNGVNVVSGPVFDFDYDGRCDSLENLRQKRRVIRNQEILIPTHFFIVLTSCKDTSQTPLHCENLDTLAFILPHRTDNSESCVHGKHDSSWVEELLMLHRARITDVEHITGLSFYQQRKEPVSDILKLKTHLPTFSQED

SEQ ID NO: 20 - protein, 1079 aa, Artificial Sequence
  chemically synthesized
MRGPAVLLTVALATLLAPGAGAPSCAKEVKSCKGRCFERTFGNCRCDAACVELGNCCLDYQETCIEPEHIWTCNKFRCGEKRLTRSLCACSDDCKDKGDCCINYSSVCQGEKSWVEEPCESINEPQCPAGFETPPTLLFSLDGFRAEYLHTWGGLLPVISKLKKCGTYTKNMRPVYPTKTFPNHYSIVTGLYPESHGIIDNKMYDPKMNASFSLKSKEKFNPEWYKGEPIWVTAKYQGLKSGTFFWPGSDVEINGIFPDIYKMYNGSVPFEERILAVLQWLQLPKDERPHFYTLYLEEPDSSGHSYGPVSSEVIKALQRVDGMVGMLMDGLKELNLHRCLNLILISDHGMEQGSCKKYIYLNKYLGDVKNIKVIYGPAARLRPSDVPDKYYSFNYEGIARNLSCREPNQHFKPYLKHFLPKRLHFAKSDRIEPLTFYLDPQWQLALNPSERKYCGSGFHGSDNVFSNMQALFVGYGPGFKHGIEADTFENIEVYNLMCDLLNLTPAPNNGTHGSLNHLLKNPVYTPKHPKEVHPLVQCPFTRNPRDNLGCSCNPSILPIEDFQTQFNLTVAEEKIIKHETLPYGRPRVLQKENTICLLSQHQFMSGYSQDILMPLWTSYTVDRNDSFSTEDFSNCLYQDFRIPLSPVHKCSFYKNNTKVSYGFLSPPQLNKNSSGIYSEALLTTNIVPMYQSFQVIWRYFHDTLLRKYAEERNGVNVVSGPVFDFDYDGRCDSLENLRQKRRVIRNQEILIPTHFFIVLTSCKDTSQTPLHCENLDTLAFILPHRTDNSESCVHGKHDSSWVEELLMLHRARITDVEHITGLSFYQQRKEPVSDILKLKTHLPTFSQEDLINDKTHTCPPCPAPELLGGPSVFLFPPKPKDTLMISRTPEVTCVVVDVSHEDPEVKFNWYVDGVEVHNAKTKPREEQYNSTYRVVSVLTVLHQDWLNGKEYKCKVSNKALPAPIEKTISKAKGQPREPQVYTLPPSREEMTKNQVSLTCLVKGFYPSDIAVEWESNGQPENNYKTTPPVLDSDGSFFLYSKLTVDKSRWQQGNVFSCSVMHEALHNHYTQKSLSLSPGK

SEQ ID NO: 21 - protein, 1550 aa, Artificial Sequence
  chemically synthesized
MERDGCAGGGSRGGEGGRAPREGPAGNGRDRGRSHAAEAPGDPQAAASLLAPMDVGEEPLEKAARARTAKDPNTYKIISLFTFAVGVNICLGFTAGLKPSCAKEVKSCKGRCFERTFGNCRCDAACVELGNCCLDYQETCIEPEHIWTCNKFRCGEKRLTRSLCACSDDCKDKGDCCINYSSVCQGEKSWVEEPCESINEPQCPAGFETPPTLLFSLDGFRAEYLHTWGGLLPVISKLKKCGTYTKNMRPVYPTKTFPNHYSIVTGLYPESHGIIDNKMYDPKMNASFSLKSKEKFNPEWYKGEPIWVTAKYQGLKSGTFFWPGSDVEINGIFPDIYKMYNGSVPFEERILAVLQWLQLPKDERPHFYTLYLEEPDSSGHSYGPVSSEVIKALQRVDGMVGMLMDGLKELNLHRCLNLILISDHGMEQGSCKKYIYLNKYLGDVKNIKVIYGPAARLRPSDVPDKYYSFNYEGIARNLSCREPNQHFKPYLKHFLPKRLHFAKSDRIEPLTFYLDPQWQLALNPSERKYCGSGFHGSDNVFSNMQALFVGYGPGFKHGIEADTFENIEVYNLMCDLLNLTPAPNNGTHGSLNHLLKNPVYTPKHPKEVHPLVQCPFTRNPRDNLGCSCNPSILPIEDFQTQFNLTVAEEKIIKHETLPYGRPRVLQKENTICLLSQHQFMSGYSQDILMPLWTSYTVDRNDSFSTEDFSNCLYQDFRIPLSPVHKCSFYKNNTKVSYGFLSPPQLNKNSSGIYSEALLTTNIVPMYQSFQVIWRYFHDTLLRKYAEERNGVNVVSGPVFDFDYDGRCDSLENLRQKRRVIRNQEILIPTHFFIVLTSCKDTSQTPLHCENLDTLAFILPHRTDNSESCVHGKHDSSWVEELLMLHRARITDVEHITGLSFYQQRKEPVSDILKLKTHLPTFSQEDRSGSGGSMKWVTFLLLLFVSGSAFSRGVFRREAHKSEIAHRYNDLGEQHFKGLVLIAFSQYLQKCSYDEHAKLVQEVTDFAKTCVADESAANCDKSLHTLFGDKLCAIPNLRENYGELADCCTKQEPERNECFLQHKDDNPSLPPFERPEAEAMCTSFKENPTTFMGHYLHEVARRHPYFYAPELLYYAEQYNEILTQCCAEADKESCLTPKLDGVKEKALVSSVRQRMKCSSMQKFGERAFKAWAVARLSQTFPNADFAEITKLATDLTKVNKECCHGDLLECADDRAELAKYMCENQATISSKLQTCCDKPLLKKAHCLSEVEHDTMPADLPAIAADFVEDQEVCKNYAEAKDVFLGTFLYEYSRRHPDYSVSLLLRLAKKYEATLEKCCAEANPPACYGTVLAEFQPLVEEPKNLVKTNCDLYEKLGEYGFQNAILVRYTQKAPQVSTPTLVEAARNLGRVGTKCCTLPEDQRLPCVEDYLSAILNRVCLLHEKTPVSEHVTKCCSGSLVERRPCFSALTVDETYVPKEFKAETFTFHSDICTLPEKEKQIKKQTALAELVKHKPKATAEQLKTVMDDFAQFLDTCCKAADKDTCFSTEGPNLVTRCKDALARSWSHPQFEK

SEQ ID NO: 22 - protein, 1474 aa, Artificial Sequence
  chemically synthesized
MRGPAVLLTVALATLLAPGAGAPSCAKEVKSCKGRCFERTFGNCRCDAACVELGNCCLDYQETCIEPEHIWTCNKFRCGEKRLTRSLCACSDDCKDKGDCCINYSSVCQGEKSWVEEPCESINEPQCPAGFETPPTLLFSLDGFRAEYLHTWGGLLPVISKLKKCGTYTKNMRPVYPTKTFPNHYSIVTGLYPESHGIIDNKMYDPKMNASFSLKSKEKFNPEWYKGEPIWVTAKYQGLKSGTFFWPGSDVEINGIFPDIYKMYNGSVPFEERILAVLQWLQLPKDERPHFYTLYLEEPDSSGHSYGPVSSEVIKALQRVDGMVGMLMDGLKELNLHRCLNLILISDHGMEQGSCKKYIYLNKYLGDVKNIKVIYGPAARLRPSDVPDKYYSFNYEGIARNLSCREPNQHFKPYLKHFLPKRLHFAKSDRIEPLTFYLDPQWQLALNPSERKYCGSGFHGSDNVFSNMQALFVGYGPGFKHGIEADTFENIEVYNLMCDLLNLTPAPNNGTHGSLNHLLKNPVYTPKHPKEVHPLVQCPFTRNPRDNLGCSCNPSILPIEDFQTQFNLTVAEEKIIKHETLPYGRPRVLQKENTICLLSQHQFMSGYSQDILMPLWTSYTVDRNDSFSTEDFSNCLYQDFRIPLSPVHKCSFYKNNTKVSYGFLSPPQLNKNSSGIYSEALLTTNIVPMYQSFQVIWRYFHDTLLRKYAEERNGVNVVSGPVFDFDYDGRCDSLENLRQKRRVIRNQEILIPTHFFIVLTSCKDTSQTPLHCENLDTLAFILPHRTDNSESCVHGKHDSSWVEELLMLHRARITDVEHITGLSFYQQRKEPVSDILKLKTHLPTFSQEDRSGSGGSMKWVTFLLLLFVSGSAFSRGVFRREAHKSEIAHRYNDLGEQHFKGLVLIAFSQYLQKCSYDEHAKLVQEVTDFAKTCVADESAANCDKSLHTLFGDKLCAIPNLRENYGELADCCTKQEPERNECFLQHKDDNPSLPPFERPEAEAMCTSFKENPTTFMGHYLHEVARRHPYFYAPELLYYAEQYNEILTQCCAEADKESCLTPKLDGVKEKALVSSVRQRMKCSSMQKFGERAFKAWAVARLSQTFPNADFAEITKLATDLTKVNKECCHGDLLECADDRAELAKYMCENQATISSKLQTCCDKPLLKKAHCLSEVEHDTMPADLPAIAADFVEDQEVCKNYAEAKDVFLGTFLYEYSRRHPDYSVSLLLRLAKKYEATLEKCCAEANPPACYGTVLAEFQPLVEEPKNLVKTNCDLYEKLGEYGFQNAILVRYTQKAPQVSTPTLVEAARNLGRVGTKCCTLPEDQRLPCVEDYLSAILNRVCLLHEKTPVSEHVTKCCSGSLVERRPCFSALTVDETYVPKEFKAETFTFHSDICTLPEKEKQIKKQTALAELVKHKPKATAEQLKTVMDDFAQFLDTCCKAADKDTCFSTEGPNLVTRCKDALARSWSHPQFEK

SEQ ID NO: 23 - protein, 19 aa, Artificial Sequence
  chemically synthesized
IISLFTFAVGVNICLGFTA

SEQ ID NO: 24 - protein, 850 aa, Artificial Sequence
  chemically synthesized
MTSKFLLVSFILAALSLSTTFSLQPSCAKEVKSCKGRCFERTFSNCRCDAACVSLGNCCLDFQETCVEPTHIWTCNKFRCGEKRLSRFVCSCADDCKTHNDCCINYSSVCQDKKSWVEETCESIDTPECPAEFESPPTLLFSLDGFRAEYLHTWGGLLPVISKLKNCGTYTKNMRPMYPTKTFPNHYSIVTGLYPESHGIIDNKMYDPKMNASFSLKSKEKFNPLWYKGQPIWVTANHQEVKSGTYFWPGSDVEIDGILPDIYKVYNGSVPFEERILAVLEWLQLPSHERPHFYTLYLEEPDSSGHSHGPVSSEVIKALQKVDRLVGMLMDGLKDLGLDKCLNLILISDHGMEQGSCKKYVYLNKYLGDVNNVKVVYGPAARLRPTDVPETYYSFNYEALAKNLSCREPNQHFRPYLKPFLPKRLHFAKSDRIEPLTFYLDPQWQLALNPSERKYCGSGFHGSDNLFSNMQALFIGYGPAFKHGAEVDSFENIEVYNLMCDLLGLIPAPNNGSHGSLNHLLKKPIYNPSHPKEEGFLSQCPIKSTSNDLGCTCDPWIVPIKDFEKQLNLTTEDVDDIYHMTVPYGRPRILLKQHRVCLLQQQQFLTGYSLDLLMPLWASYTFLSNDQFSRDDFSNCLYQDLRIPLSPVHKCSYYKSNSKLSYGFLTPPRLNRVSNHIYSEALLTSNIVPMYQSFQVIWHYLHDTLLQRYAHERNGINVVSGPVFDFDYDGRYDSLEILKQNSRVIRSQEILIPTHFFIVLTSCKQLSETPLECSALESSAYILPHRPDNIESCTHGKRESSWVEELLTLHRARVTDVELITGLSFYQDRQESVSELLRLKTHLPIFSQED

SEQ ID NO: 25 - protein, 1474 aa, Artificial Sequence
  chemically synthesized
MTSKFLLVSFILAALSLSTTFSLQPSCAKEVKSCKGRCFERTFSNCRCDAACVSLGNCCLDFQETCVEPTHIWTCNKFRCGEKRLSRFVCSCADDCKTHNDCCINYSSVCQDKKSWVEETCESIDTPECPAEFESPPTLLFSLDGFRAEYLHTWGGLLPVISKLKNCGTYTKNMRPMYPTKTFPNHYSIVTGLYPESHGIIDNKMYDPKMNASFSLKSKEKFNPLWYKGQPIWVTANHQEVKSGTYFWPGSDVEIDGILPDIYKVYNGSVPFEERILAVLEWLQLPSHERPHFYTLYLEEPDSSGHSHGPVSSEVIKALQKVDRLVGMLMDGLKDLGLDKCLNLILISDHGMEQGSCKKYVYLNKYLGDVNNVKVVYGPAARLRPTDVPETYYSFNYEALAKNLSCREPNQHFRPYLKPFLPKRLHFAKSDRIEPLTFYLDPQWQLALNPSERKYCGSGFHGSDNLFSNMQALFIGYGPAFKHGAEVDSFENIEVYNLMCDLLGLIPAPNNGSHGSLNHLLKKPIYNPSHPKEEGFLSQCPIKSTSNDLGCTCDPWIVPIKDFEKQLNLTTEDVDDIYHMTVPYGRPRILLKQHRVCLLQQQQFLTGYSLDLLMPLWASYTFLSNDQFSRDDFSNCLYQDLRIPLSPVHKCSYYKSNSKLSYGFLTPPRLNRVSNHIYSEALLTSNIVPMYQSFQVIWHYLHDTLLQRYAHERNGINVVSGPVFDFDYDGRYDSLEILKQNSRVIRSQEILIPTHFFIVLTSCKQLSETPLECSALESSAYILPHRPDNIESCTHGKRESSWVEELLTLHRARVTDVELITGLSFYQDRQESVSELLRLKTHLPIFSQEDGGSGGSMKWVTFLLLLFVSGSAFSRGVFRREAHKSEIAHRYNDLGEQHFKGLVLIAFSQYLQKCSYDEHAKLVQEVTDFAKTCVADESAANCDKSLHTLFGDKLCAIPNLRENYGELADCCTKQEPERNECFLQHKDDNPSLPPFERPEAEAMCTSFKENPTTFMGHYLHEVARRHPYFYAPELLYYAEQYNEILTQCCAEADKESCLTPKLDGVKEKALVSSVRQRMKCSSMQKFGERAFKAWAVARLSQTFPNADFAEITKLATDLTKVNKECCHGDLLECADDRAELAKYMCENQATISSKLQTCCDKPLLKKAHCLSEVEHDTMPADLPAIAADFVEDQEVCKNYAEAKDVFLGTFLYEYSRRHPDYSVSLLLRLAKKYEATLEKCCAEANPPACYGTVLAEFQPLVEEPKNLVKTNCDLYEKLGEYGFQNAILVRYTQKAPQVSTPTLVEAARNLGRVGTKCCTLPEDQRLPCVEDYLSAILNRVCLLHEKTPVSEHVTKCCSGSLVERRPCFSALTVDETYVPKEFKAETFTFHSDICTLPEKEKQIKKQTALAELVKHKPKATAEQLKTVMDDFAQFLDTCCKAADKDTCFSTEGPNLVTRCKDALARSWSHPQFEK

SEQ ID NO: 26 - protein, 227 aa, Artificial Sequence
  chemically synthesized
DKTHTCPPCPAPELLGGPSVFLFPPKPKDTLMISRTPEVTCVVVDVSHEDPEVKFNWYVDGVEVHNAKTKPREEQYNSTYRVVSVLTVLHQDWLNGKEYKCKVSNKALPAPIEKTISKAKGQPREPQVYTLPPSREEMTKNQVSLTCLVKGFYPSDIAVEWESNGQPENNYKTTPPVLDSDGSFFLYSKLTVDKSRWQQGNVFSCSVMHEALHNHYTQKSLSLSPGK

SEQ ID NO: 27 - protein, 618 aa, Artificial Sequence
  chemically synthesized
MKWVTFLLLLFVSGSAFSRGVFRREAHKSEIAHRYNDLGEQHFKGLVLIAFSQYLQKCSYDEHAKLVQEVTDFAKTCVADESAANCDKSLHTLFGDKLCAIPNLRENYGELADCCTKQEPERNECFLQHKDDNPSLPPFERPEAEAMCTSFKENPTTFMGHYLHEVARRHPYFYAPELLYYAEQYNEILTQCCAEADKESCLTPKLDGVKEKALVSSVRQRMKCSSMQKFGERAFKAWAVARLSQTFPNADFAEITKLATDLTKVNKECCHGDLLECADDRAELAKYMCENQATISSKLQTCCDKPLLKKAHCLSEVEHDTMPADLPAIAADFVEDQEVCKNYAEAKDVFLGTFLYEYSRRHPDYSVSLLLRLAKKYEATLEKCCAEANPPACYGTVLAEFQPLVEEPKNLVKTNCDLYEKLGEYGFQNAILVRYTQKAPQVSTPTLVEAARNLGRVGTKCCTLPEDQRLPCVEDYLSAILNRVCLLHEKTPVSEHVTKCCSGSLVERRPCFSALTVDETYVPKEFKAETFTFHSDICTLPEKEKQIKKQTALAELVKHKPKATAEQLKTVMDDFAQFLDTCCKAADKDTCFSTEGPNLVTRCKDALARSWSHPQFEK

SEQ ID NO: 28 - protein, 3 aa, Artificial Sequence
  chemically synthesized
LIN

SEQ ID NO: 29 - protein, 6 aa, Artificial Sequence
  chemically synthesized
GGSGGS

SEQ ID NO: 30 - protein, 7 aa, Artificial Sequence
  chemically synthesized
RSGSGGS